European Patent Application EP 4 538 395 A2, published April 16, 2025. Title: METHODS AND COMPOSITIONS FOR RECOMBINASE-MEDIATED SELECTED CLEAVAGE OF NUCLEIC ACIDS. Applicant: ILLUMINA, INC. Application WO PCT/US2019/022443, filed March 15, 2019. The sequence listing filed with the application follows.

SEQUENCE LISTING (11 sequences)

SEQ ID NO: 1 - protein, 196 aa, synthetic construct
QLVKSELEEKKSELRHKLKYVPHEYIELIEIARNSTQDRILEMKVMEFFMKVYGYRGKHLGGSRKPDGAIYTVGSPIDYGVIVDTKAYSGGYNLPIGQADEMQRYVEENQTRNKHINPNEWWKVYPSSVTEFKFLFVSGHFKGNYKAQLTRLNHITNCNGAVLSVEELLIGGEMIKAGTLTLEEVRRKFNNGEINF

SEQ ID NO: 2 - protein, 196 aa, synthetic construct
QLVKSELEEKKSELRHKLKYVPHEYIELIEIARNSTQDRILEMKVMEFFMKVYGYRGKHLGGSRKPDGAIYTVGSPIDYGVIVDTKAYSGGYNLPIGQADEMERYVEENQTRNKHLNPNEWWKVYPSSVTEFKFLFVSGHFKGNYKAQLTRLNHITNCNGAVLSVEELLIGGEMIKAGTLTLEEVRRKFNNGEINF

SEQ ID NO: 3 - protein, 196 aa, synthetic construct
QLVKSELEEKKSELRHKLKYVPHEYIELIEIARNSTQDRILEMKVMEFFMKVYGYRGKHLGGSRKPDGAIYTVGSPIDYGVIVDTKAYSGGYNLPIGQADEMQRYVKENQTRNKHINPNEWWKVYPSSVTEFKFLFVSGHFKGNYKAQLTRLNHKTNCNGAVLSVEELLIGGEMIKAGTLTLEEVRRKFNNGEINF

SEQ ID NO: 4 - protein, 196 aa, synthetic construct
QLVKSELEEKKSELRHKLKYVPHEYIELIEIARNSTQDRILEMKVMEFFMKVYGYRGKHLGGSRKPDGAIYTVGSPIDYGVIVDTKAYSGGYNLPIGQADEMQDYVEENQTRNKHINPNEWWKVYPSSVTEFKFLFVSGHFKGNYKAQLTRLNHITNCNGAVLSVEELLIGGEMIKAGTLTLEEVRRKFNNGEINF

SEQ ID NO: 5 - protein, 196 aa, synthetic construct
QLVKSELEEKKSELRHKLKYVPHEYIELIEIARNSTQDRILEMKVMEFFMKVYGYRGKHLGGSRKPDGAIYTVGSPIDYGVIVDTKAYSGGYNLPIGQAREMQRYVEENQTRNKHINPNEWWKVYPSSVTEFKFLFVSGHFKGNYKAQLTRLNHITNCNGAVLSVEELLIGGEMIKAGTLTLEEVRRKFNNGEINF

SEQ ID NO: 6 - protein, 196 aa, synthetic construct
QLVKSELEEKKSELRHKLKYVPHEYIELIEIARNSTQDRILEMKVMEFFMKVYGYRGKHLGGSRKPDGAIYTVGSPIDYGVIVDTKAYSGGYNLPIGQADEMERYVEENQTRNKHANPNEWWKVYPSSVTEFKFLFVSGHFKGNYKAQLTRLNHITNCNGAVLSVEELLIGGEMIKAGTLTLEEVRRKFNNGEINF

SEQ ID NO: 7 - protein, 196 aa, synthetic construct
QLVKSELEEKKSELRHKLKYVPHEYIELIEIARNSTQDRILEMKVMEFFMKVYGYRGKHLGGSRKPDGAIYTVGSPIDYGVIVDTKAYSGGYNLPIGQADEMQRYVKENQTRNKHINPNEWWKVYPSSVTEFKFLFVSGHFKGNYKAQLTRLNHVTNCNGAVLSVEELLIGGEMIKAGTLTLEEVRRKFNNGEINF

SEQ ID NO: 8 - protein, 196 aa, synthetic construct
QLVKSELEEKKSELRHKLKYVPHEYIELIEIARNSTQDRILEMKVMEFFMKVYGYRGKHLGGSRKPDGAIYTVGSPIDYGVIVDTKAYSGGYNLPIGQADEMERYVEENQTRDKHLNPNEWWKVYPSSVTEFKFLFVSGHFKGNYKAQLTRLNHITNCNGAVLSVEELLIGGEMIKAGTLTLEEVRRKFNNGEINF

SEQ ID NO: 9 - protein, 196 aa, synthetic construct
QLVKSELEEKKSELRHKLKYVPHEYIELIEIARNSTQDRILEMKVMEFFMKVYGYRGKHLGGSRKPDGAIYTVGSPIDYGVIVDTKAYSGGYNLPIGQADEMQRYVKENQTRNKHINPNEWWKVYPSSVTEFKFLFVSGHFKGNYKAQLTRLNRKTNCNGAVLSVEELLIGGEMIKAGTLTLEEVRRKFNNGEINF

SEQ ID NO: 10 - protein, 196 aa, synthetic construct
QLVKSELEEKKSELRHKLKYVPHEYIELIEIARNPTQDRILEMKVMEFFMKVYGYRGEHLGGSRKPDGAIYTVGSPIDYGVIVDTKAYSGGYNLPIGQADEMQRYVEENQTRNKHINPNEWWKVYPSSVTEFKFLFVSGHFKGNYKAQLTRLNHITNCNGAVLSVEELLIGGEMIKAGTLTLEEVRRKFNNGEINF

SEQ ID NO: 11 - protein, 196 aa, synthetic construct
QLVKSELEEKKSELRHKLKYVPHEYIELIEIARNPTQDRILEMKVMEFLMKVYGYRGEHLGGSRKPDGAIYTVGSPIDYGVIVDTKAYSGGYNLPIGHADEMQRYVEENQTRNKHINPNEWWKVYPSSVTEFKFLFVSGYFKGDYKAQLTRLNHITNCNGAVLSVEELLIGGEMIQAGTLTLEEVRRKFNNGEINF